European Patent Application EP 4 534 098 A1, published April 9, 2025. Title: Oral vaccine composition. Applicant: KAICO LTD. The sequence listing filed with the application follows.

SEQUENCE LISTING (2 sequences)

SEQ ID NO: 1 - DNA, 705 bp, synthetic construct
  misc_feature 1..705: note = Synthetic DNA
  source 1..705: mol_type = other DNA
  CDS 1..705
atgggcacttatccgaggaggcgttaccgcagaagaagacacagaccccgtagtcacctgggacaaatactcagaaggagaccgtggctggtccacccgcgtcataggtatagatggagacgcaaaaacggaatcttcaatacgaggctgagcagaacttttggctacaccgtcaaggcaacaactgtacgcactccgtcctgggcggtcgacatgatgcgtttcaacattgacgattttgtacctccaggtggaggcaccaacaaaatctcgattcccttcgaatactatcgcattcgtaaagtgaaggttgagttttggccttgctcgccaataacgcaaggtgaccgtggtgtgggaagtacagctgttatcctggacgataacttcgtgaccaaggctacggccttgacatacgatccttatgttaattactcatctaggcacacaattcctcaaccattcagctatcattcccgctactttacgccgaaacccgtactcgactctacaatcgattacttccagccaaacaataagagaactcaactgtggttgcgcctccagacctcacgtaacgtcgaccacgtaggcctgggtactgcctttgaaaactctatctacgaccaagattacaacatcagggtgaccatgtacgttcagttcagagagttcaacctcaaggatccgccccttaagccttaa

SEQ ID NO: 2 - protein, 234 aa, synthetic construct
  REGION 1..234: note = Synthetic Construct
MGTYPRRRYRRRRHRPRSHLGQILRRRPWLVHPRHRYRWRRKNGIFNTRLSRTFGYTVKATTVRTPSWAVDMMRFNIDDFVPPGGGTNKISIPFEYYRIRKVKVEFWPCSPITQGDRGVGSTAVILDDNFVTKATALTYDPYVNYSSRHTIPQPFSYHSRYFTPKPVLDSTIDYFQPNNKRTQLWLRLQTSRNVDHVGLGTAFENSIYDQDYNIRVTMYVQFREFNLKDPPLKP